European Patent Specification EP 3 697 917 B1, published May 15, 2024. Title: Vectors. Applicant: Oxford Genetics Limited. The sequence listing filed with the application follows.

SEQUENCE LISTING (21 sequences)

SEQ ID NO: 1 - DNA, 1866 bp, adeno-associated virus 2
atgccggggttttacgagattgtgattaaggtccccagcgaccttgacgagcatctgcccggcatttctgacagctttgtgaactgggtggccgagaaggaatgggagttgccgccagattctgacatggatctgaatctgattgagcaggcacccctgaccgtggccgagaagctgcagcgcgactttctgacggaatggcgccgtgtgagtaaggccccggaggcccttttctttgtgcaatttgagaagggagagagctacttccacatgcacgtgctcgtggaaaccaccggggtgaaatccatggttttgggacgtttcctgagtcagattcgcgaaaaactgattcagagaatttaccgcgggatcgagccgactttgccaaactggttcgcggtcacaaagaccagaaatggcgccggaggcgggaacaaggtggtggatgagtgctacatccccaattacttgctccccaaaacccagcctgagctccagtgggcgtggactaatatggaacagtatttaagcgcctgtttgaatctcacggagcgtaaacggttggtggcgcagcatctgacgcacgtgtcgcagacgcaggagcagaacaaagagaatcagaatcccaattctgatgcgccggtgatcagatcaaaaacttcagccaggtacatggagctggtcgggtggctcgtggacaaggggattacctcggagaagcagtggatccaggaggaccaggcctcatacatctccttcaatgcggcctccaactcgcggtcccaaatcaaggctgccttggacaatgcgggaaagattatgagcctgactaaaaccgcccccgactacctggtgggccagcagcccgtggaggacatttccagcaatcggatttataaaattttggaactaaacgggtacgatccccaatatgcggcttccgtctttctgggatgggccacgaaaaagttcggcaagaggaacaccatctggctgtttgggcctgcaactaccgggaagaccaacatcgcggaggccatagcccacactgtgcccttctacgggtgcgtaaactggaccaatgagaactttcccttcaacgactgtgtcgacaagatggtgatctggtgggaggaggggaagatgaccgccaaggtcgtggagtcggccaaagccattctcggaggaagcaaggtgcgcgtggaccagaaatgcaagtcctcggcccagatagacccgactcccgtgatcgtcacctccaacaccaacatgtgcgccgtgattgacgggaactcaacgaccttcgaacaccagcagccgttgcaagaccggatgttcaaatttgaactcacccgccgtctggatcatgactttgggaaggtcaccaagcaggaagtcaaagactttttccggtgggcaaaggatcacgtggttgaggtggagcatgaattctacgtcaaaaagggtggagccaagaaaagacccgcccccagtgacgcagatataagtgagcccaaacgggtgcgcgagtcagttgcgcagccatcgacgtcagacgcggaagcttcgatcaactacgcagacaggtaccaaaacaaatgttctcgtcacgtgggcatgaatctgatgctgtttccctgcagacaatgcgagagaatgaatcagaattcaaatatctgcttcactcacggacagaaagactgtttagagtgctttcccgtgtcagaatctcaacccgtttctgtcgtcaaaaaggcgtatcagaaactgtgctacattcatcatatcatgggaaaggtgccagacgcttgcactgcctgcgatctggtcaatgtggatttggatgactgcatctttgaacaatag

SEQ ID NO: 2 - protein, 621 aa, adeno-associated virus 2
MPGFYEIVIKVPSDLDGHLPGISDSFVNWVAEKEWELPPDSDMDLNLIEQAPLTVAEKLQRDFLTEWRRVSKAPEALFFVQFEKGESYFHMHVLVETTGVKSMVLGRFLSQIREKLIQRIYRGIEPTLPNWFAVTKTRNGAGGGNKVVDECYIPNYLLPKTQPELQWAWTNMEQYLSACLNLTERKRLVAQHLTHVSQTQEQNKENQNPNSDAPVIRSKTSARYMELVGWLVDKGITSEKQWIQEDQASYISFNAASNSRSQIKAALDNAGKIMSLTKTAPDYLVGQQPVEDISSNRIYKILELNGYDPQYAASVFLGWATKKFGKRNTIWLFGPATTGKTNIAEAIAHTVPFYGCVNWTNENFPFNDCVDKMVIWWEEGKMTAKVVESAKAILGGSKVRVDQKCKSSAQIDPTPVIVTSNTNMCAVIDGNSTTFEHQQPLQDRMFKFELTRRLDHDFGKVTKQEVKDFFRWAKDHVVEVEHEFYVKKGGAKKRPAPSDADISEPKRVRESVAQPSTSDAEASINYADRYQNKCSRHVGMNLMLFPCRQCERMNQNSNICFTHGQKDCLECFPVSESQPVSVVKKAYQKLCYIHHIMGKVPDACTACDLVNVDLDDCIFEQ

SEQ ID NO: 3 - protein, 528 aa, adeno-associated virus 2
MPGFYEIVIKVPSDLDEHLPGISDSFVNWVAEKEWELPPDSDMDLNLIEQAPLTVAEKLQRDFLTEWRRVSKAPEALFFVQFEKGESYFHMHVLVETTGVKSMVLGRFLSQIREKLIQRIYRGIEPTLPNWFAVTKTRNGAGGGNKVVDECYIPNYLLPKTQPELQWAWTNMEQYLSACLNLTERKRLVAQHLTHVSQTQEQNKENQNPNSDAPVIRSKTSARYMELVGWLVDKGITSEKQWIQEDQASYISFNAASNSRSQIKAALDNAGKIMSLTKTAPDYLVGQQPVEDISSNRIYKILELNGYDPQYAASVFLGWATKKFGKRNTIWLFGPATTGKTNIAEAIAHTVPFYGCVNWTNENFPFNDCVDKMVIWWEEGKMTAKVVESAKAILGGSKVRVDQKCKSSAQIDPTPVIVTSNTNMCAVIDGNSTTFEHQQPLQDRMFKFELTRRLDHDFGKVTKQEVKDFFRWAKDHVVEVEHEFYVKKGGAKKRPAPSDADISEPKRVRESVAQPSTSDAEASINYAD

SEQ ID NO: 4 - protein, 397 aa, adeno-associated virus 2
MELVGWLVDKGITSEKQWIQEDQASYISFNAASNSRSQIKAALDNAGKIMSLTKTAPDYLVGQQPVEDISSNRIYKILELNGYDPQYAASVFLGWATKKFGKRNTIWLFGPATTGKTNIAEAIAHTVPFYGCVNWTNENFPFNDCVDKMVIWWEEGKMTAKVVESAKAILGGSKVRVDQKCKSSAQIDPTPVIVTSNTNMCAVIDGNSTTFEHQQPLQDRMFKFELTRRLDHDFGKVTKQEVKDFFRWAKDHVVEVEHEFYVKKGGAKKRPAPSDADISEPKRVRESVAQPSTSDAEASINYADRYQNKCSRHVGMNLMLFPCRQCERMNQNSNICFTHGQKDCLECFPVSESQPVSVVKKAYQKLCYIHHIMGKVPDACTACDLVNVDLDDCIFEQ

SEQ ID NO: 5 - protein, 312 aa, adeno-associated virus 2
MELVGWLVDKGITSEKQWIQEDQASYISFNAASNSRSQIKAALDNAGKIMSLTKTAPDYLVGQQPVEDISSNRIYKILELNGYDPQYAASVFLGWATKKFGKRNTIWLFGPATTGKTNIAEAIAHTVPFYGCVNWTNENFPFNDCVDKMVIWWEEGKMTAKVVESAKAILGGSKVRVDQKCKSSAQIDPTPVIVTSNTNMCAVIDGNSTTFEHQQPLQDRMFKFELTRRLDHDFGKVTKQEVKDFFRWAKDHVVEVEHEFYVKKGGAKKRPAPSDADISEPKRVRESVAQPSTSDAEASINYADRLARGHSL

SEQ ID NO: 6 - DNA, 1866 bp, adeno-associated virus 2
atgccggggttttacgagattgtgattaaggtccccagcgaccttgacgggcatctgcccggcatttctgacagctttgtgaactgggtggccgagaaggaatgggagttgccgccagattctgacatggatctgaatctgattgagcaggcacccctgaccgtggccgagaagctgcagcgcgactttctgacggaatggcgccgtgtgagtaaggccccggaggcccttttctttgtgcaatttgagaagggagagagctacttccacatgcacgtgctcgtggaaaccaccggggtgaaatccatggttttgggacgtttcctgagtcagattcgcgaaaaactgattcagagaatttaccgcgggatcgagccgactttgccaaactggttcgcggtcacaaagaccagaaatggcgccggaggcgggaacaaggtggtggatgagtgctacatccccaattacttgctccccaaaacccagcctgagctccagtgggcgtggactaatatggaacagtacctcagcgcctgtttgaatctcacggagcgtaaacggttggtggcgcagcatctgacgcacgtgtcgcagacgcaggagcagaacaaagagaatcagaatcccaattctgatgcgccggtgatcagatcaaaaacttcagccaggtacatggagctggtcgggtggctcgtggacaaggggattacctcggagaagcagtggatccaggaggaccaggcctcatacatctccttcaatgcggcctccaactcgcggtcccaaatcaaggctgccttggacaatgcgggaaagattatgagcctgactaaaaccgcccccgactacctggtgggccagcagcccgtggaggacatttccagcaatcggatttataaaattttggaactaaacgggtacgatccccaatatgcggcttccgtctttctgggatgggccacgaaaaagttcggcaagaggaacaccatctggctgtttgggcctgcaactaccgggaagaccaacatcgcggaggccatagcccacactgtgcccttctacgggtgcgtaaactggaccaatgagaactttcccttcaacgactgtgtcgacaagatggtgatctggtgggaggaggggaagatgaccgccaaggtcgtggagtcggccaaagccattctcggaggaagcaaggtgcgcgtggaccagaaatgcaagtcctcggcccagatagacccgactcccgtgatcgtcacctccaacaccaacatgtgcgccgtgattgacgggaactcaacgaccttcgaacaccagcagccgttgcaagaccggatgttcaaatttgaactcacccgccgtctggatcatgactttgggaaggtcaccaagcaggaagtcaaagactttttccggtgggcaaaggatcacgtggttgaggtggagcatgaattctacgtcaaaaagggtggagccaagaaaagacccgcccccagtgacgcagatataagtgagcccaaacgggtgcgcgagtcagttgcgcagccatcgacgtcagacgcggaagcttcgatcaactacgcagacaggtaccaaaacaaatgttctcgtcacgtgggcatgaatctgatgctgtttccctgcagacaatgcgagagaatgaatcagaattcaaatatctgcttcactcacggacagaaagactgtttagagtgctttcccgtgtcagaatctcaacccgtttctgtcgtcaaaaaggcgtatcagaaactgtgctacattcatcatatcatgggaaaggtgccagacgcttgcactgcctgcgatctggtcaatgtggatttggatgactgcatctttgaacaatag

SEQ ID NO: 7 - DNA, 1589 bp, adeno-associated virus 2
atgccggggttttacgagattgtgattaaggtccccagcgaccttgacgagcatctgcccggcatttctgacagctttgtgaactgggtggccgagaaggaatgggagttgccgccagattctgacatggatctgaatctgattgagcaggcacccctgaccgtggccgagaagctgcagcgcgactttctgacggaatggcgccgtgtgagtaaggccccggaggcccttttctttgtgcaatttgagaagggagagagctacttccacatgcacgtgctcgtggaaaccaccggggtgaaatccatggttttgggacgtttcctgagtcagattcgcgaaaaactgattcagagaatttaccgcgggatcgagccgactttgccaaactggttcgcggtcacaaagaccagaaatggcgccggaggcgggaacaaggtggtggatgagtgctacatccccaattacttgctccccaaaacccagcctgagctccagtgggcgtggactaatatggaacagtacctcagcgcctgtttgaatctcacggagcgtaaacggttggtggcgcagcatctgacgcacgtgtcgcagacgcaggagcagaacaaagagaatcagaatcccaattctgatgcgccggtgatcagatcaaaaacttcagccaggtacatggagctggtcgggtggctcgtggacaaggggattacctcggagaagcagtggatccaggaggaccaggcctcatacatctccttcaatgcggcctccaactcgcggtcccaaatcaaggctgccttggacaatgcgggaaagattatgagcctgactaaaaccgcccccgactacctggtgggccagcagcccgtggaggacatttccagcaatcggatttataaaattttggaactaaacgggtacgatccccaatatgcggcttccgtctttctgggatgggccacgaaaaagttcggcaagaggaacaccatctggctgtttgggcctgcaactaccgggaagaccaacatcgcggaggccatagcccacactgtgcccttctacgggtgcgtaaactggaccaatgagaactttcccttcaacgactgtgtcgacaagatggtgatctggtgggaggaggggaagatgaccgccaaggtcgtggagtcggccaaagccattctcggaggaagcaaggtgcgcgtggaccagaaatgcaagtcctcggcccagatagacccgactcccgtgatcgtcacctccaacaccaacatgtgcgccgtgattgacgggaactcaacgaccttcgaacaccagcagccgttgcaagaccggatgttcaaatttgaactcacccgccgtctggatcatgactttgggaaggtcaccaagcaggaagtcaaagactttttccggtgggcaaaggatcacgtggttgaggtggagcatgaattctacgtcaaaaagggtggagccaagaaaagacccgcccccagtgacgcagatataagtgagcccaaacgggtgcgcgagtcagttgcgcagccatcgacgtcagacgcggaagcttcgatcaactacgcagacagtag

SEQ ID NO: 8 - DNA, 1195 bp, adeno-associated virus 2
catggagctggtcgggtggctcgtggacaaggggattacctcggagaagcagtggatccaggaggaccaggcctcatacatctccttcaatgcggcctccaactcgcggtcccaaatcaaggctgccttggacaatgcgggaaagattatgagcctgactaaaaccgcccccgactacctggtgggccagcagcccgtggaggacatttccagcaatcggatttataaaattttggaactaaacgggtacgatccccaatatgcggcttccgtctttctgggatgggccacgaaaaagttcggcaagaggaacaccatctggctgtttgggcctgcaactaccgggaagaccaacatcgcggaggccatagcccacactgtgcccttctacgggtgcgtaaactggaccaatgagaactttcccttcaacgactgtgtcgacaagatggtgatctggtgggaggaggggaagatgaccgccaaggtcgtggagtcggccaaagccattctcggaggaagcaaggtgcgcgtggaccagaaatgcaagtcctcggcccagatagacccgactcccgtgatcgtcacctccaacaccaacatgtgcgccgtgattgacgggaactcaacgaccttcgaacaccagcagccgttgcaagaccggatgttcaaatttgaactcacccgccgtctggatcatgactttgggaaggtcaccaagcaggaagtcaaagactttttccggtgggcaaaggatcacgtggttgaggtggagcatgaattctacgtcaaaaagggtggagccaagaaaagacccgcccccagtgacgcagatataagtgagcccaaacgggtgcgcgagtcagttgcgcagccatcgacgtcagacgcggaagcttcgatcaactacgcagacaggtaccaaaacaaatgttctcgtcacgtgggcatgaatctgatgctgtttccctgcagacaatgcgagagaatgaatcagaattcaaatatctgcttcactcacggacagaaagactgtttagagtgctttcccgtgtcagaatctcaacccgtttctgtcgtcaaaaaggcgtatcagaaactgtgctacattcatcatatcatgggaaaggtgccagacgcttgcactgcctgcgatctggtcaatgtggatttggatgactgcatctttgaacaatag

SEQ ID NO: 9 - DNA, 939 bp, adeno-associated virus 2
atggagctggtcgggtggctcgtggacaaggggattacctcggagaagcagtggatccaggaggaccaggcctcatacatctccttcaatgcggcctccaactcgcggtcccaaatcaaggctgccttggacaatgcgggaaagattatgagcctgactaaaaccgcccccgactacctggtgggccagcagcccgtggaggacatttccagcaatcggatttataaaattttggaactaaacgggtacgatccccaatatgcggcttccgtctttctgggatgggccacgaaaaagttcggcaagaggaacaccatctggctgtttgggcctgcaactaccgggaagaccaacatcgcggaggccatagcccacactgtgcccttctacgggtgcgtaaactggaccaatgagaactttcccttcaacgactgtgtcgacaagatggtgatctggtgggaggaggggaagatgaccgccaaggtcgtggagtcggccaaagccattctcggaggaagcaaggtgcgcgtggaccagaaatgcaagtcctcggcccagatagacccgactcccgtgatcgtcacctccaacaccaacatgtgcgccgtgattgacgggaactcaacgaccttcgaacaccagcagccgttgcaagaccggatgttcaaatttgaactcacccgccgtctggatcatgactttgggaaggtcaccaagcaggaagtcaaagactttttccggtgggcaaaggatcacgtggttgaggtggagcatgaattctacgtcaaaaagggtggagccaagaaaagacccgcccccagtgacgcagatataagtgagcccaaacgggtgcgcgagtcagttgcgcagccatcgacgtcagacgcggaagcttcgatcaactacgcagacagattggctcgaggacactctctctag

SEQ ID NO: 10 - DNA, 2559 bp, adeno-associated virus 2
cagttgcgcagccatcgacgtcagacgcggaagcttcgatcaactacgcagacaggtaccaaaacaaatgttctcgtcacgtgggcatgaatctgatgctgtttccctgcagacaatgcgagagaatgaatcagaattcaaatatctgcttcactcacggacagaaagactgtttagagtgctttcccgtgtcagaatctcaacccgtttctgtcgtcaaaaaggcgtatcagaaactgtgctacattcatcatatcatgggaaaggtgccagacgcttgcactgcctgcgatctggtcaatgtggatttggatgactgcatctttgaacaataaatgatttaaatcaggtatggctgccgatggttatcttccagattggctcgaggacactctctctgaaggaataagacagtggtggaagctcaaacctggcccaccaccaccaaagcccgcagagcggcataaggacgacagcaggggtcttgtgcttcctgggtacaagtacctcggacccttcaacggactcgacaagggagagccggtcaacgaggcagacgccgcggccctcgagcacgacaaagcctacgaccggcagctcgacagcggagacaacccgtacctcaagtacaaccacgccgacgcggagtttcaggagcgccttaaagaagatacgtcttttgggggcaacctcggacgagcagtcttccaggcgaaaaagagggttcttgaacctctgggcctggttgaggaacctgttaagacggctccgggaaaaaagaggccggtagagcactctcctgtggagccagactcctcctcgggaaccggaaaggcgggccagcagcctgcaagaaaaagattgaattttggtcagactggagacgcagactcagtacctgacccccagcctctcggacagccaccagcagccccctctggtctgggaactaatacgatggctacaggcagtggcgcaccaatggcagacaataacgagggcgccgacggagtgggtaattcctcgggaaattggcattgcgattccacatggatgggcgacagagtcatcaccaccagcacccgaacctgggccctgcccacctacaacaaccacctctacaaacaaatttccagccaatcaggagcctcgaacgacaatcactactttggctacagcaccccttgggggtattttgacttcaacagattccactgccacttttcaccacgtgactggcaaagactcatcaacaacaactggggattccgacccaagagactcaacttcaagctctttaacattcaagtcaaagaggtcacgcagaatgacggtacgacgacgattgccaataaccttaccagcacggttcaggtgtttactgactcggagtaccagctcccgtacgtcctcggctcggcgcatcaaggatgcctcccgccgttcccagcagacgtcttcatggtgccacagtatggatacctcaccctgaacaacgggagtcaggcagtaggacgctcttcattttactgcctggagtactttccttctcagatgctgcgtaccggaaacaactttaccttcagctacacttttgaggacgttcctttccacagcagctacgctcacagccagagtctggaccgtctcatgaatcctctcatcgaccagtacctgtattacttgagcagaacaaacactccaagtggaaccaccacgcagtcaaggcttcagttttctcaggccggagcgagtgacattcgggaccagtctaggaactggcttcctggaccctgttaccgccagcagcgagtatcaaagacatctgcggataacaacaacagtgaatactcgtggactggagctaccaagtaccacctcaatggcagagactctctggtgaatccgggcccggccatggcaagccacaaggacgatgaagaaaagttttttcctcagagcggggttctcatctttgggaagcaaggctcagagaaaacaaatgtggacattgaaaaggtcatgattacagacgaagaggaaatcaggacaaccaatcccgtggctacggagcagtatggttctgtatctaccaacctccagagaggcaacagacaagcagctaccgcagatgtcaacacacaaggcgttcttccaggcatggtctggcaggacagagatgtgtaccttcaggggcccatctgggcaaagattccacacacggacggacattttcacccctctcccctcatgggtggattcggacttaaacaccctcctccacagattctcatcaagaacaccccggtacctgcgaatccttcgaccaccttcagtgcggcaaagtttgcttccttcatcacacagtactccacgggacaggtcagcgtggagatcgagtgggagctgcagaaggaaaacagcaaacgctggaatcccgaaattcagtacacttccaactacaacaagtctgttaatgtggactttactgtggacactaatggcgtgtattcagagcctcgccccattggcaccagatacctgactcgtaatctgtaa

SEQ ID NO: 11 - protein, 735 aa, adeno-associated virus 2 [sequence omitted]

SEQ ID NO: 12 - DNA, 19 bp, Artificial Sequence
  TetR binding site
tccctatcagtgatagaga

SEQ ID NO: 13 - DNA, 624 bp, Artificial Sequence
  Nucleotide sequence of the TetR protein
atgtcgcgcctggacaaaagcaaagtgattaactcagcgctggaactgttgaatgaggtgggaattgaaggactcactactcgcaagctggcacagaagctgggcgtcgagcagccaacgctgtactggcatgtgaagaataaacgggcgctcctagacgcgcttgccatcgaaatgctggaccgccatcacacccacttttgccccctggagggcgaatcctggcaagattttctgcggaacaatgcaaagtcgttccggtgcgctctgctgtcccaccgcgatggcgcaaaagtgcacctgggcactcggcccaccgagaaacaatacgaaaccctggaaaaccaactggctttcctttgccaacagggattttcactggagaatgccctgtacgcactatccgcggtcggccactttaccctgggatgcgtcctcgaagatcaggagcaccaagtcgccaaggaggaaagagaaactcctaccactgactcaatgcctccgctcctgagacaagccatcgagctgttcgaccaccagggtgctgaacctgcatttctgttcgggcttgaactgattatctgcggcctggagaaacagttgaagtgcgagtcgggatcctag

SEQ ID NO: 14 - protein, 207 aa, Artificial Sequence
  Amino acid sequence of the TetR protein
MSRLDKSKVINSALELLNEVGIEGLTTRKLAQKLGVEQPTLYWHVKNKRALLDALAIEMLDRHHTHFCPLEGESWQDFLRNNAKSFRCALLSHRDGAKVHLGTRPTEKQYETLENQLAFLCQQGFSLENALYALSAVGHFTLGCVLEDQEHQVAKEERETPTTDSMPPLLRQAIELFDHQGAEPAFLFGLELIICGLEKQLKCESGS

SEQ ID NO: 15 - DNA, 519 bp, Encephalomyocarditis virus
cgttactggccgaagccgcttggaataaggccggtgtgcgtttgtctatatgttattttccaccatattgccgtcttttggcaatgtgagggcccggaaacctggccctgtcttcttgacgagcattcctaggggtctttcccctctcgccaaaggaatgcaaggtctgttgaatgtcgtgaaggaagcagttcctctggaagcttcttgaagacaaacaacgtctgtagcgaccctttgcaggcagcggaaccccccacctggcgacaggtgcctctgcggccaaaagccacgtgtataagatacacctgcaaaggcggcacaaccccagtgccacgttgtgagttggatagttgtggaaagagtcaaatggctcccctcaagcgtattcaacaaggggctgaaggatgcccagaaggtaccccattgtatgggatctgatctggggcctcggtgcacatgctttacatgtgtttagtcgaggttaaaaaacgtctaggccccccgaaccacggggac

SEQ ID NO: 16 - DNA, 461 bp, Foot-and-mouth disease virus
agcaggtttccccaactgacacaaaacgtgcaacttgaaactccgcctggtctttccaggtctagaggggtaacactttgtactgcgtttggctccacgctcgatccactggcgagtgttagtaacagcactgttgcttcgtagcggagcatgacggccgtgggaactcctccttggtaacaaggacccacggggccaaaagccacgcccacacgggcccgtcatgtgtgcaaccccagcacggcgactttactgcgaaacccactttaaagtgacattgaaactggtacccacacactggtgacaggctaaggatgcccttcaggtaccccgaggtaacacgcgacactcgggatctgagaaggggactggggcttctataaaagcgctcggtttaaaaagcttctatgcctgaataggtgaccggaggtcggcacctttcctttgcaattactgaccac

SEQ ID NO: 17 - DNA, 5341 bp, Human adenovirus type 5
ggtacccaactccatgctcaacagtccccaggtacagcccaccctgcgtcgcaaccaggaacagctctacagcttcctggagcgccactcgccctacttccgcagccacagtgcgcagattaggagcgccacttctttttgtcacttgaaaaacatgtaaaaataatgtactagagacactttcaataaaggcaaatgcttttatttgtacactctcgggtgattatttacccccacccttgccgtctgcgccgtttaaaaatcaaaggggttctgccgcgcatcgctatgcgccactggcagggacacgttgcgatactggtgtttagtgctccacttaaactcaggcacaaccatccgcggcagctcggtgaagttttcactccacaggctgcgcaccatcaccaacgcgtttagcaggtcgggcgccgatatcttgaagtcgcagttggggcctccgccctgcgcgcgcgagttgcgatacacagggttgcagcactggaacactatcagcgccgggtggtgcacgctggccagcacgctcttgtcggagatcagatccgcgtccaggtcctccgcgttgctcagggcgaacggagtcaactttggtagctgccttcccaaaaagggcgcgtgcccaggctttgagttgcactcgcaccgtagtggcatcaaaaggtgaccgtgcccggtctgggcgttaggatacagcgcctgcataaaagccttgatctgcttaaaagccacctgagcctttgcgccttcagagaagaacatgccgcaagacttgccggaaaactgattggccggacaggccgcgtcgtgcacgcagcaccttgcgtcggtgttggagatctgcaccacatttcggccccaccggttcttcacgatcttggccttgctagactgctccttcagcgcgcgctgcccgttttcgctcgtcacatccatttcaatcacgtgctccttatttatcataatgcttccgtgtagacacttaagctcgccttcgatctcagcgcagcggtgcagccacaacgcgcagcccgtgggctcgtgatgcttgtaggtcacctctgcaaacgactgcaggtacgcctgcaggaatcgccccatcatcgtcacaaaggtcttgttgctggtgaaggtcagctgcaacccgcggtgctcctcgttcagccaggtcttgcatacggccgccagagcttccacttggtcaggcagtagtttgaagttcgcctttagatcgttatccacgtggtacttgtccatcagcgcgcgcgcagcctccatgcccttctcccacgcagacacgatcggcacactcagcgggttcatcaccgtaatttcactttccgcttcgctgggctcttcctcttcctcttgcgtccgcataccacgcgccactgggtcgtcttcattcagccgccgcactgtgcgcttacctcctttgccatgcttgattagcaccggtgggttgctgaaacccaccatttgtagcgccacatcttctctttcttcctcgctgtccacgattacctctggtgatggcgggcgctcgggcttgggagaagggcgcttctttttcttcttgggcgcaatggccaaatccgccgccgaggtcgatggccgcgggctgggtgtgcgcggcaccagcgcgtcttgtgatgagtcttcctcgtcctcggactcgatacgccgcctcatccgcttttttgggggcgcccggggaggcggcggcgacggggacggggacgacacgtcctccatggttgggggacgtcgcgccgcaccgcgtccgcgctcgggggtggtttcgcgctgctcctcttcccgactggccatttccttctcctataggcagaaaaagatcatggagtcagtcgagaagaaggacagcctaaccgccccctctgagttcgccaccaccgcctccaccgatgccgccaacgcgcctaccaccttccccgtcgaggcacccccgcttgaggaggaggaagtgattatcgagcaggacccaggttttgtaagcgaagacgacgaggaccgctcagtaccaacagaggataaaaagcaagaccaggacaacgcagaggcaaacgaggaacaagtcgggcggggggacgaaaggcatggcgactacctagatgtgggagacgacgtgctgttgaagcatctgcagcgccagtgcgccattatctgcgacgcgttgcaagagcgcagcgatgtgcccctcgccatagcggatgtcagccttgcctacgaacgccacctattctcaccgcgcgtaccccccaaacgccaagaaaacggcacatgcgagcccaacccgcgcctcaacttctaccccgtatttgccgtgccagaggtgcttgccacctatcacatctttttccaaaactgcaagatacccctatcctgccgtgccaaccgcagccgagcggacaagcagctggccttgcggcagggcgctgtcatacctgatatcgcctcgctcaacgaagtgccaaaaatctttgagggtcttggacgcgacgagaagcgcgcggcaaacgctctgcaacaggaaaacagcgaaaatgaaagtcactctggagtgttggtggaactcgagggtgacaacgcgcgcctagccgtactaaaacgcagcatcgaggtcacccactttgcctacccggcacttaacctaccccccaaggtcatgagcacagtcatgagtgagctgatcgtgcgccgtgcgcagcccctggagagggatgcaaatttgcaagaacaaacagaggagggcctacccgcagttggcgacgagcagctagcgcgctggcttcaaacgcgcgagcctgccgacttggaggagcgacgcaaactaatgatggccgcagtgctcgttaccgtggagcttgagtgcatgcagcggttctttgctgacccggagatgcagcgcaagctagaggaaacattgcactacacctttcgacagggctacgtacgccaggcctgcaagatctccaacgtggagctctgcaacctggtctcctaccttggaattttgcacgaaaaccgccttgggcaaaacgtgcttcattccacgctcaagggcgaggcgcgccgcgactacgtccgcgactgcgtttacttatttctatgctacacctggcagacggccatgggcgtttggcagcagtgcttggaggagtgcaacctcaaggagctgcagaaactgctaaagcaaaacttgaaggacctatggacggccttcaacgagcgctccgtggccgcgcacctggcggacatcattttccccgaacgcctgcttaaaaccctgcaacagggtctgccagacttcaccagtcaaagcatgttgcagaactttaggaactttatcctagagcgctcaggaatcttgcccgccacctgctgtgcacttcctagcgactttgtgcccattaagtaccgcgaatgccctccgccgctttggggccactgctaccttctgcagctagccaactaccttgcctaccactctgacataatggaagacgtgagcggtgacggtctactggagtgtcactgtcgctgcaacctatgcaccccgcaccgctccctggtttgcaattcgcagctgcttaacgaaagtcaaattatcggtacctttgagctgcagggtccctcgcctgacgaaaagtccgcggctccggggttgaaactcactccggggctgtggacgtcggcttaccttcgcaaatttgtacctgaggactaccacgcccacgagattaggttctacgaagaccaatcccgcccgcctaatgcggagcttaccgcctgcgtcattacccagggccacattcttggccaattgcaagccatcaacaaagcccgccaagagtttctgctacgaaagggacggggggtttacttggacccccagtccggcgaggagctcaacccaatccccccgccgccgcagccctatcagcagcagccgcgggcccttgcttcccaggatggcacccaaaaagaagctgcagctgccgccgccacccacggacgaggaggaatactgggacagtcaggcagaggaggttttggacgaggaggaggaggacatgatggaagactgggagagcctagacgaggaagcttccgaggtcgaagaggtgtcagacgaaacaccgtcaccctcggtcgcattcccctcgccggcgccccagaaatcggcaaccggttccagcatggctacaacctccgctcctcaggcgccgccggcactgcccgttcgccgacccaaccgtagatgggacaccactggaaccagggccggtaagtccaagcagccgccgccgttagcccaagagcaacaacagcgccaaggctaccgctcatggcgcgggcacaagaacgccatagttgcttgcttgcaagactgtgggggcaacatctccttcgcccgccgctttcttctctaccatcacggcgtggccttcccccgtaacatcctgcattactaccgtcatctctacagcccatactgcaccggcggcagcggcagcaacagcagcggccacacagaagcaaaggcgaccggatagcaagactctgacaaagcccaagaaatccacagcggcggcagcagcaggaggaggagcgctgcgtctggcgcccaacgaacccgtatcgacccgcgagcttagaaacaggatttttcccactctgtatgctatatttcaacagagcaggggccaagaacaagagctgaaaataaaaaacaggtctctgcgatccctcacccgcagctgcctgtatcacaaaagcgaagatcagcttcggcgcacgctggaagacgcggaggctctcttcagtaaatactgcgcgctgactcttaaggactagtttcgcgccctttctcaaatttaagcgcgaaaactacgtcatctccagcggccacacccggcgccagcacctgttgtcagcgccattatgagcaaggaaattcccacgccctacatgtggagttaccagccacaaatgggacttgcggctggagctgcccaagactactcaacccgaataaactacatgagcgcgggaccccacatgatatcccgggtcaacggaatacgcgcccaccgaaaccgaattcccttggaacaggcggctattaccaccacacctcgtaataaccttaatccccgtagttggcccgctgccctggtgtaccaggaaagtcccgctcccaccactgtggtacttcccagagacgcccaggccgaagttcagatgactaactcaggggcgcagcttgcgggcggctttcgtcacagggtgcggtcgcccgggc

SEQ ID NO: 18 - DNA, 573 bp, Cytomegalovirus genus
agtaatcaattacggggtcattagttcatagcccatatatggagttccgcgttacataacttacggtaaatggcccgcctggctgaccgcccaacgacccccgcccattgacgtcaataatgacgtatgttcccatagtaacgccaatagggactttccattgacgtcaatgggtggagtatttacggtaaactgcccacttggcagtacatcaagtgtatcatatgccaagtacgccccctattgacgtcaatgacggtaaatggcccgcctggcattatgcccagtacatgaccttatgggactttcctacttggcagtacatctacgtattagtcatcgctattaccatgctgatgcggttttggcagtacatcaatgggcgtggatagcggtttgactcacggggatttccaagtctccaccccattgacgtcaatgggagtttgttttggcaccaaaatcaacgggactttccaaaatgtcgtaacaactccgccccattgacgcaaatgggcggtaggcgtgtacggtgggaggtctatataagcagagctggtttagtgaaccgtc

SEQ ID NO: 19 - DNA, 637 bp, Artificial Sequence
  CMV promoter inducible (p565-2xTetO)
cgtgaggctccggtgcccgtcagtgggcagagcgcacatcgcccacagtccccgagaagttggggggaggggtcggcaattgaaccggtgcctagagaaggtggcgcggggtaaactgggaaagtgatgtcgtgtactggctccgcctttttcccgagggtgggggagaaccgtatataagtgcactagtcgccgtgaacgtcaatggaaagtccctattggcgttactatgggaacatacgtcattattgacgtcaatgacggtaaatggcccgcctggcattatgcccagtacatgaccttatgggactttcctacttggcagtacatctacgtattagtcatcgctattaccatgctgatgcggttttggcagtacatcaatgggcgtggatagcggtttgactcacggggatttccaagtctccaccccattgacgtcaatgggagtttgttttggcaccaaaatcaacgggactttccaaaatgtcgtaacaactccgccccattgacgcaaatgggcggtaggcgtgtacggtgggaggtctatataagcagagctgtccctatcagtgatagagatgtccctatcagtgatagagatcgtcgagcagctcgtttagtgaaccgtcagatc

SEQ ID NO: 20 - DNA, 2559 bp, adeno-associated virus 2; identical to SEQ ID NO: 10

SEQ ID NO: 21 - DNA, 192 bp, Simian virus 40
cagacatgataagatacattgatgagtttggacaaaccacaactagaatgcagtgaaaaaaatgctttatttgtgaaatttgtgatgctattgctttatttgtaaccattataagctgcaataaacaagttaacaacaacaattgcattcattttatgtttcaggttcagggggaggtgtgggaggtttttt